European Patent Application EP 4 617 290 A1, published September 17, 2025. Title: ANTIBODY AND USE THEREOF. Applicant: SICHUAN HUIYU PHARMACEUTICAL CO., LTD. The sequence listing filed with the application follows.

SEQUENCE LISTING (88 sequences)

SEQ ID NO: 1 - protein, 115 aa, synthetic construct
  source 1..115: note = VHH amino acid sequence of 3C6hu-1
EVQLVESGGGLIQPGGSLRLSCAASGNIGSIRHMGWVRQAPGKGLEWVSTITTVGTTYYANFVKGRFTISRDNSKNTLYLQMNSLRAEDTAVYYCRATAHPTDYWGQGTLVTVSS

SEQ ID NO: 2 - protein, 115 aa, synthetic construct
  source 1..115: note = VHH amino acid sequence of 3C6hu-2
EVQLVESGGGLIQPGGSLRLSCAASGNIGSIRHMGWHRQAPGKGLELVSTITTVGTTYYANFVKGRFTISRDNSKNTLYLQMNSLRAEDTAVYYCRATAHPTDYWGQGTLVTVSS

SEQ ID NO: 3 - protein, 115 aa, synthetic construct
  source 1..115: note = VHH amino acid sequence of 3C6hu-3
EVQLVESGGGLIQPGGSLRLSCAASGNIGSIRHMGWHRQAPGKELELVSTITTVGTTYYANFVKGRFTISRDNSKNTLYLQMNSLRAEDTAVYYCRATAHPTDYWGQGTLVTVSS

SEQ ID NO: 4 - protein, 115 aa, synthetic construct
  source 1..115: note = VHH amino acid sequence of 3C6hu-4
EVQLVESGGGLIQPGGSLRLSCAASGNIGSIRHMGWHRQAPGKGRELVSTITTVGTTYYANFVKGRFTISRDNSKNTLYLQMNSLRAEDTAVYYCRATAHPTDYWGQGTLVTVSS

SEQ ID NO: 5 - protein, 115 aa, synthetic construct
  source 1..115: note = VHH amino acid sequence of 3C6hu-5
EVQLVESGGGLIQPGGSLRLSCAASGNIGSIRHMGWHRQAPGKERELVSTITTVGTTYYANFVKGRFTISRDNSKNTLYLQMNSLRAEDTAVYYCRATAHPTDYWGQGTLVTVSS

SEQ ID NO: 6 - protein, 115 aa, synthetic construct
  source 1..115: note = VHH amino acid sequence of 3C6hu-6
EVQLVESGGGLIQPGGSLRLSCAASGNIGSIRHMGWHRQAPGKERELVATITTVGTTYYANFVKGRFTISRDNSKNTLYLQMNSLRAEDTAVYYCRATAHPTDYWGQGTLVTVSS

SEQ ID NO: 7 - protein, 115 aa, synthetic construct
  source 1..115: note = VHH amino acid sequence of 3C6hu-7
EVQLVESGGGLIQPGGSLRLSCAASGNIGSIRHMGWHRQAPGKEREWVATITTVGTTYYANFVKGRFTISRDNSKNTLYLQMNSLRAEDTAVYYCRATAHPTDYWGQGTLVTVSS

SEQ ID NO: 8 - protein, 115 aa, synthetic construct
  source 1..115: note = VHH amino acid sequence of 3C6hu-8
EVQLVESGGGLIQPGGSLRLSCAASGNIGSIRHMGWVRQAPGKERELVATITTVGTTYYANFVKGRFTISRDNSKNTLYLQMNSLRAEDTAVYYCRATAHPTDYWGQGTLVTVSS

SEQ ID NO: 9 - protein, 115 aa, synthetic construct
  source 1..115: note = 3C6
EVQLVESGGGLVQAGESLRLSCAVSGNIGSIRHMGWHRQDPGKERELVATITTVGTTYYANFVKGRFTISRDNAKNTVYLQMNSLKPEDTGVYYCRATAHPTDYWGQGTQVTVSS

SEQ ID NO: 10 - protein, 123 aa, synthetic construct
  source 1..123: note = 4A7
EVQLVESGGGLVQAGDSLRLGCAASGRTFSTNVMGWFRQAPGKEREFVSAISRAGSTYSADSVKGRFTISRDNAENTVYLQMNSLKPEDTAVYYCAAGSSPTAIFGKSGMDYWGKGTLVTVSS

SEQ ID NO: 11 - protein, 8 aa, synthetic construct
  source 1..8: note = 4A7 CDR1-1(IMGT)
GRTFSTNV

SEQ ID NO: 12 - protein, 7 aa, synthetic construct
  source 1..7: note = 4A7 CDR2(IMGT)
ISRAGST

SEQ ID NO: 13 - protein, 17 aa, synthetic construct
  source 1..17: note = 4A7 CDR3(IMGT)
AAGSSPTAIFGKSGMDY

SEQ ID NO: 14 - protein, 5 aa, synthetic construct
  source 1..5: note = 4A7 CDR1(Kabat)
TNVMG

SEQ ID NO: 15 - protein, 16 aa, synthetic construct
  source 1..16: note = 4A7 CDR2(Kabat)
AISRAGSTYSADSVKG

SEQ ID NO: 16 - protein, 15 aa, synthetic construct
  source 1..15: note = 4A7 CDR3(Kabat/ AbM/Chothia)
GSSPTAIFGKSGMDY

SEQ ID NO: 17 - protein, 10 aa, synthetic construct
  source 1..10: note = 4A7 CDR1(AbM)
GRTFSTNVMG

SEQ ID NO: 18 - protein, 9 aa, synthetic construct
  source 1..9: note = 4A7 CDR2(AbM)
AISRAGSTY

SEQ ID NO: 19 - protein, 7 aa, synthetic construct
  source 1..7: note = 4A7 CDR1(Chothia)
GRTFSTN

SEQ ID NO: 20 - protein, 5 aa, synthetic construct
  source 1..5: note = 4A7 CDR2(Chothia)
SRAGS

SEQ ID NO: 21 - protein, 6 aa, synthetic construct
  source 1..6: note = 4A7 CDR1(Contact)
STNVMG

SEQ ID NO: 22 - protein, 12 aa, synthetic construct
  source 1..12: note = 4A7 CDR2(Contact)
FVSAISRAGSTY

SEQ ID NO: 23 - protein, 16 aa, synthetic construct
  source 1..16: note = 4A7 CDR3(Contact)
AAGSSPTAIFGKSGMD

SEQ ID NO: 24 - protein, 123 aa, synthetic construct
  source 1..123: note = VHH amino acid sequence of 4A7hu-1
EVQLLESGGGLVQPGGSLRLSCAASGRTFSTNVMSWVRQAPGKGLEWVSAISRAGSTYYADSVKGRFTISRDNSKNTLYLQMNSLRAEDTAVYYCAAGSSPTAIFGKSGMDYWGQGTQVTVSS

SEQ ID NO: 25 - protein, 123 aa, synthetic construct
  source 1..123: note = VHH amino acid sequence of 4A7hu-2
EVQLLESGGGLVQPGGSLRLSCAASGRTFSTNVMGWVRQAPGKGLEWVSAISRAGSTYSADSVKGRFTISRDNSKNTLYLQMNSLRAEDTAVYYCAAGSSPTAIFGKSGMDYWGQGTQVTVSS

SEQ ID NO: 26 - protein, 123 aa, synthetic construct
  source 1..123: note = VHH amino acid sequence of 4A7hu-3
EVQLLESGGGLVQPGGSLRLSCAASGRTFSTNVMGWFRQAPGKGLEWVSAISRAGSTYSADSVKGRFTISRDNSKNTLYLQMNSLRAEDTAVYYCAAGSSPTAIFGKSGMDYWGQGTQVTVSS

SEQ ID NO: 27 - protein, 123 aa, synthetic construct
  source 1..123: note = VHH amino acid sequence of 4A7hu-4
EVQLLESGGGLVQPGGSLRLSCAASGRTFSTNVMGWVRQAPGKGLEFVSAISRAGSTYSADSVKGRFTISRDNSKNTLYLQMNSLRAEDTAVYYCAAGSSPTAIFGKSGMDYWGQGTQVTVSS

SEQ ID NO: 28 - protein, 123 aa, synthetic construct
  source 1..123: note = VHH amino acid sequence of 4A7hu-5
EVQLLESGGGLVQPGGSLRLSCAASGRTFSTNVMGWFRQAPGKGLEFVSAISRAGSTYSADSVKGRFTISRDNSKNTLYLQMNSLRAEDTAVYYCAAGSSPTAIFGKSGMDYWGQGTQVTVSS

SEQ ID NO: 29 - protein, 123 aa, synthetic construct
  source 1..123: note = VHH amino acid sequence of 4A7hu-6
EVQLLESGGGLVQAGGSLRLSCAASGRTFSTNVMGWFRQAPGKGLEFVSAISRAGSTYSADSVKGRFTISRDNSKNTLYLQMNSLRAEDTAVYYCAAGSSPTAIFGKSGMDYWGQGTQVTVSS

SEQ ID NO: 30 - protein, 123 aa, synthetic construct
  source 1..123: note = VHH amino acid sequence of 4A7hu-7
EVQLLESGGGLVQPGGSLRLSCAASGRTFSTNVMGWFRQAPGKGREFVSAISRAGSTYSADSVKGRFTISRDNSKNTLYLQMNSLRAEDTAVYYCAAGSSPTAIFGKSGMDYWGQGTQVTVSS

SEQ ID NO: 31 - protein, 123 aa, synthetic construct
  source 1..123: note = VHH amino acid sequence of 4A7hu-8
EVQLLESGGGLVQPGGSLRLSCAASGRTFSTNVMGWFRQAPGKEREFVSAISRAGSTYSADSVKGRFTISRDNSKNTLYLQMNSLRAEDTAVYYCAAGSSPTAIFGKSGMDYWGQGTQVTVSS

SEQ ID NO: 32 - protein, 123 aa, synthetic construct
  source 1..123: note = VHH amino acid sequence of 4A7hu-9
EVQLLESGGGLVQPGGSLRLSCAASGRTFSSYVMSWVRQAPGKGLEWVSAISRAGSTYYADSVKGRFTISRDNSKNTLYLQMNSLRAEDTAVYYCAAGSSPTAIFGKSGMDYWGQGTQVTVSS

SEQ ID NO: 33 - protein, 123 aa, synthetic construct
  source 1..123: note = VHH amino acid sequence of 4A7hu-10
EVQLLESGGGLVQPGGSLRLSCAASGRTFSSYVMGWVRQAPGKGLEWVSAISRAGSTYSADSVKGRFTISRDNSKNTLYLQMNSLRAEDTAVYYCAAGSSPTAIFGKSGMDYWGQGTQVTVSS

SEQ ID NO: 34 - protein, 123 aa, synthetic construct
  source 1..123: note = VHH amino acid sequence of 4A7hu-11
EVQLLESGGGLVQPGGSLRLSCAASGRTFSSYVMGWFRQAPGKGLEWVSAISRAGSTYSADSVKGRFTISRDNSKNTLYLQMNSLRAEDTAVYYCAAGSSPTAIFGKSGMDYWGQGTQVTVSS

SEQ ID NO: 35 - protein, 123 aa, synthetic construct
  source 1..123: note = VHH amino acid sequence of 4A7hu-12
EVQLLESGGGLVQPGGSLRLSCAASGRTFSSYVMGWVRQAPGKGLEFVSAISRAGSTYSADSVKGRFTISRDNSKNTLYLQMNSLRAEDTAVYYCAAGSSPTAIFGKSGMDYWGQGTQVTVSS

SEQ ID NO: 36 - protein, 123 aa, synthetic construct
  source 1..123: note = VHH amino acid sequence of 4A7hu-13
EVQLLESGGGLVQPGGSLRLSCAASGRTFSSYVMGWFRQAPGKGLEFVSAISRAGSTYSADSVKGRFTISRDNSKNTLYLQMNSLRAEDTAVYYCAAGSSPTAIFGKSGMDYWGQGTQVTVSS

SEQ ID NO: 37 - protein, 123 aa, synthetic construct
  source 1..123: note = VHH amino acid sequence of 4A7hu-14
EVQLLESGGGLVQAGGSLRLSCAASGRTFSSYVMGWFRQAPGKGLEFVSAISRAGSTYSADSVKGRFTISRDNSKNTLYLQMNSLRAEDTAVYYCAAGSSPTAIFGKSGMDYWGQGTQVTVSS

SEQ ID NO: 38 - protein, 123 aa, synthetic construct
  source 1..123: note = VHH amino acid sequence of 4A7hu-15
EVQLLESGGGLVQPGGSLRLSCAASGRTFSSYVMGWFRQAPGKGREFVSAISRAGSTYSADSVKGRFTISRDNSKNTLYLQMNSLRAEDTAVYYCAAGSSPTAIFGKSGMDYWGQGTQVTVSS

SEQ ID NO: 39 - protein, 123 aa, synthetic construct
  source 1..123: note = VHH amino acid sequence of 4A7hu-16
EVQLLESGGGLVQPGGSLRLSCAASGRTFSSYVMGWFRQAPGKEREFVSAISRAGSTYSADSVKGRFTISRDNSKNTLYLQMNSLRAEDTAVYYCAAGSSPTAIFGKSGMDYWGQGTQVTVSS

SEQ ID NO: 40 - protein, 125 aa, synthetic construct
  source 1..125: note = CD3-VH1
EVQLVESGGGLVQPGGSLRLSCAASGFTFNTYAMNWVRQAPGKGLEWVARIRSKYNNYATYYADSVKGRFTISRDDSKSSLYLQMNSLKTEDTAVYYCVRHGNFGNNYVSWFASWGQGTLVTVSS

SEQ ID NO: 41 - protein, 125 aa, synthetic construct
  source 1..125: note = CD3-VH2
EVQLVESGGGLVQPGGSLRLSCAASGFTFNTYAMNWVRQAPGKGLEWVARIRSKYNNYATYYADSVKGRFTISRDDSKSILYLQMNSLKTEDTAMYYCVRHERFGNSYVSWFAYWGQGTLVTVSS

SEQ ID NO: 42 - protein, 125 aa, synthetic construct
  source 1..125: note = CD3-VH3
EVQLVESGGGLVQPGGSLRLSCAASGFTFNTYAMNWVRQAPGKGLEWVARIRSKYNNYATYYADSVKDRFTISRDDSKSSLYLQMNNLKTEDTAMYYCVRHGNFGNTYVSWFAMWGQGTLVTVSS

SEQ ID NO: 43 - protein, 109 aa, synthetic construct
  source 1..109: note = CD3-VL
QAVVTQEPSFSVSPGGTVTLTCRSSTGAVTTSNYANWVQQTPGQAFRGLIGGTNKRAPGVPARFSGSLIGDKAALTITGAQADDESIYFCALWYSNLWVFGGGTKLTVL

SEQ ID NO: 44 - protein, 106 aa, synthetic construct
  source 1..106: note = Light chain constant region
GQPKAAPSVTLFPPSSEELQANKATLVCLISDFYPGAVTVAWKADSSPVKAGVETTTPSKQSNNKYAASSYLSLTPEQWKSHRSYSCQVTHEGSTVEKTVAPTECS

SEQ ID NO: 45 - protein, 329 aa, synthetic construct
  source 1..329: note = Mutant 1 of IgG1
ASTKGPSVFPLAPSSKSTSGGTAALGCLVKDYFPEPVTVSWNSGALTSGVHTFPAVLQSSGLYSLSSVVTVPSSSLGTQTYICNVNHKPSNTKVDKKVEPKSCDKTHTCPPCPAPEAAGAPSVFLFPPKPKDTLMISRTPEVTCVVVDVSHEDPEVKFNWYVDGVEVHNAKTKPREEQYNSTYRVVSVLTVLHQDWLNGKEYKCAVSNKALPAPIEKTISKAKGQPREPQVYTLPPSRDELTKNQVSLWCLVKGFYPSDIAVEWESNGQPENNYKTTPPVLDSDGSFFLYSKLTVDKSRWQQGNVFSCSVMHEALHNHYTQKSLSLSPG

SEQ ID NO: 46 - protein, 226 aa, synthetic construct
  source 1..226: note = Mutant 1-Fc of IgG1
DKTHTCPPCPAPEAAGAPSVFLFPPKPKDTLMISRTPEVTCVVVDVSHEDPEVKFNWYVDGVEVHNAKTKPREEQYNSTYRVVSVLTVLHQDWLNGKEYKCAVSNKALPAPIEKTISKAKGQPREPQVYTLPPSRDELTKNQVSLWCLVKGFYPSDIAVEWESNGQPENNYKTTPPVLDSDGSFFLYSKLTVDKSRWQQGNVFSCSVMHEALHNHYTQKSLSLSPG

SEQ ID NO: 47 - protein, 226 aa, synthetic construct
  source 1..226: note = Mutant 2-Fc of IgG1
DKTHTCPPCPAPEAAGAPSVFLFPPKPKDTLMISRTPEVTCVVVDVSHEDPEVKFNWYVDGVEVHNAKTKPREEQYNSTYRVVSVLTVLHQDWLNGKEYKCAVSNKALPAPIEKTISKAKGQPREPQVYTLPPSRDELTKNQVSLSCAVKGFYPSDIAVEWESNGQPENNYKTTPPVLDSDGSFFLVSKLTVDKSRWQQGNVFSCSVMHEALHNHYTQKSLSLSPG

SEQ ID NO: 48 - protein, 225 aa, synthetic construct
  source 1..225: note = Human IgG1 Fc
DKTHTCPPCPAPEAAGAPSVFLFPPKPKDTLMISRTPEVTCVVVDVSHEDPEVKFNWYVDGVEVHNAKTKPREEQYNSTYRVVSVLTVLHQDWLNGKEYKCAVSNKALPAPIEKTISKAKGQPREPQVYTLPPSRDELTKNQVSLTCLVKGFYPSDIAVEWESNGQPENNYKTTPPVLDSDGSFFLYSKLTVDKSRWQQGNVFSCSVMHEALHNHYTQKSLSLSP

SEQ ID NO: 49 - protein, 5 aa, synthetic construct
  source 1..5: note = Linker-1
GGGGS

SEQ ID NO: 50 - protein, 10 aa, synthetic construct
  source 1..10: note = Linker-2
GGGGSGGGGS

SEQ ID NO: 51 - protein, 15 aa, synthetic construct
  source 1..15: note = Linker-3
GGGGSGGGGSGGGGS

SEQ ID NO: 52 - protein, 8 aa, synthetic construct
  source 1..8: note = 3C6 CDR1(IMGT)
GNIGSIRH

SEQ ID NO: 53 - protein, 7 aa, synthetic construct
  source 1..7: note = 3C6 CDR2(IMGT)
ITTVGTT

SEQ ID NO: 54 - protein, 9 aa, synthetic construct
  source 1..9: note = 3C6 CDR3(IMGT)
RATAHPTDY

SEQ ID NO: 55 - protein, 5 aa, synthetic construct
  source 1..5: note = CD3 HCDR1(Kabat)
TYAMN

SEQ ID NO: 56 - protein, 15 aa, synthetic construct
  source 1..15: note = CD3 HCDR2(Kabat)
IRSKYNNYATYYADS

SEQ ID NO: 57 - protein, 14 aa, synthetic construct
  source 1..14: note = CD3 HCDR3-1(Kabat)
HGNFGNNYVSWFAS

SEQ ID NO: 58 - protein, 14 aa, synthetic construct
  source 1..14: note = CD3 HCDR3-2(Kabat)
HERFGNSYVSWFAY

SEQ ID NO: 59 - protein, 14 aa, synthetic construct
  source 1..14: note = CD3 HCDR3-3(Kabat)
HGNFGNTYVSWFAM

SEQ ID NO: 60 - protein, 13 aa, synthetic construct
  source 1..13: note = CD3 LCDR1(Kabat)
SSTGAVTTSNYAN

SEQ ID NO: 61 - protein, 7 aa, synthetic construct
  source 1..7: note = CD3 LCDR2(Kabat)
GTNKRAP

SEQ ID NO: 62 - protein, 8 aa, synthetic construct
  source 1..8: note = CD3 LCDR3(Kabat)
LWYSNLWV

SEQ ID NO: 63 - protein, 8 aa, synthetic construct
  source 1..8: note = 4A7 CDR1-2(IMGT)
GRTFSSYV

SEQ ID NO: 64 - protein, 125 aa, synthetic construct
  source 1..125: note = CD3-VH4
EVQLVESGGGLVQPGGSLRLSCAASGFTFNTYAMNWVRQAPGKGLEWVARIRSKYNNYATYYADSVKGRFTISRDDSKSSLYLQMNSLKTEDTAVYYCVRHGNFKNSYGSWFAYWGQGTLVTVSS

SEQ ID NO: 65 - protein, 14 aa, synthetic construct
  source 1..14: note = CD3 HCDR3-4(Kabat)
HGNFKNSYGSWFAY

SEQ ID NO: 66 - protein, 509 aa, synthetic construct
  source 1..509: note = Control antibody
QVQLVESGGGVVQAGGSLTLSCAASGSTFSIRAMRWYRQAPGTERDLVAVIYGSSTYYADAVKGRFTISRDNSKNTLYLQMNSLRAEDTAVYYCNADTIGTARDYWGQGTLVTVSSGGGGSGGGSEVQLVESGGGLVQPGNSLRLSCAASGFTFSKFGMSWVRQAPGKGLEWVSSISGSGRDTLYADSVKGRFTISRDNAKTTLYLQMNSLRPEDTAVYYCTIGGSLSVSSQGTLVTVSSGGGGSGGGSEVQLVESGGGLVQPGGSLKLSCAASGFTFNKYAINWVRQAPGKGLEWVARIRSKYNNYATYYADQVKDRFTISRDDSKNTAYLQMNNLKTEDTAVYYCVRHANFGNSYISYWAYWGQGTLVTVSSGGGGSGGGGSGGGGSQTVVTQEPSLTVSPGGTVTLTCASSTGAVTSGNYPNWVQQKPGQAPRGLIGGTKFLVPGTPARFSGSLLGGKAALTLSGVQPEDEAEYYCTLWYSNRWVFGGGTKLTVLGGSHHHHHHHH

SEQ ID NO: 67 - protein, 124 aa, synthetic construct
  source 1..124: note = 260-7-B11
EVQLVESGGGLVQAGGSLRLSCAASGGTFLTYGMGWFRQAPGKEREFVAAINWSGSMTNYADSVKGRSTISRDNARNTVYLQMISLKPEDTAVYYCAAKTGAVAYIQKNEYDYWGQGTQVTVSS

SEQ ID NO: 68 - protein, 8 aa, synthetic construct
  source 1..8: note = IMGT 260-7-B11 CDR1
GGTFLTYG

SEQ ID NO: 69 - protein, 8 aa, synthetic construct
  source 1..8: note = IMGT 260-7-B11 CDR2
INWSGSMT

SEQ ID NO: 70 - protein, 17 aa, synthetic construct
  source 1..17: note = IMGT 260-7-B11 CDR3
AAKTGAVAYIQKNEYDY

SEQ ID NO: 71 - protein, 5 aa, synthetic construct
  source 1..5: note = Kabat 260-7-B11 CDR1
TYGMG

SEQ ID NO: 72 - protein, 17 aa, synthetic construct
  source 1..17: note = Kabat 260-7-B11 CDR2
AINWSGSMTNYADSVKG

SEQ ID NO: 73 - protein, 15 aa, synthetic construct
  source 1..15: note = Kabat/ AbM/ Chothia 260-7-B11 CDR3
KTGAVAYIQKNEYDY

SEQ ID NO: 74 - protein, 10 aa, synthetic construct
  source 1..10: note = AbM 260-7-B11 CDR1
GGTFLTYGMG

SEQ ID NO: 75 - protein, 10 aa, synthetic construct
  source 1..10: note = AbM 260-7-B11 CDR2
AINWSGSMTN

SEQ ID NO: 76 - protein, 7 aa, synthetic construct
  source 1..7: note = Chothia 260-7-B11 CDR1
GGTFLTY

SEQ ID NO: 77 - protein, 6 aa, synthetic construct
  source 1..6: note = Chothia 260-7-B11 CDR2
NWSGSM

SEQ ID NO: 78 - protein, 6 aa, synthetic construct
  source 1..6: note = Contact 260-7-B11 CDR1
LTYGMG

SEQ ID NO: 79 - protein, 13 aa, synthetic construct
  source 1..13: note = Contact 260-7-B11 CDR2
FVAAINWSGSMTN

SEQ ID NO: 80 - protein, 16 aa, synthetic construct
  source 1..16: note = Contact 260-7-B11 CDR3
AAKTGAVAYIQKNEYD

SEQ ID NO: 81 - protein, 124 aa, synthetic construct
  source 1..124: note = VHH amino acid sequence of 7B11_huGS_HM4
EVQLVESGGGLVQPGGSLRLSCAASGGTFLTYGMGWFRQAPGKGLEFVAAINWSGSMTNYADSVKGRFTISRDNAKNTVYLQMNSLRAEDTAVYYCAAKTGAVAYIQKNEYDYWGQGTQVTVSS

SEQ ID NO: 82 - protein, 124 aa, synthetic construct
  source 1..124: note = VHH amino acid sequence of 7B11_huBSM1
EVQLVESGGGLVQAGGSLRLSCAASGGTFLTYGMGWFRQAPGKERVFVAAINWSGSMTNYADSVKGRFTISRDNAKNTVYLQMRSLTSEDTAVYYCAAKTGAVAYIQKNEYDYWGQGTQVTVSS

SEQ ID NO: 83 - protein, 124 aa, synthetic construct
  source 1..124: note = VHH amino acid sequence of 7B11_huBSM_HM1
EVQLVESGGGLVQAGGSLRLSCAASGGTFLTYGMGWFRQAPGKGLVFVAAINWSGSMTNYADSVKGRFTISRDNAKNTVYLQMRSLTSEDTAVYYCAAKTGAVAYIQKNEYDYWGQGTQVTVSS

SEQ ID NO: 84 - protein, 124 aa, synthetic construct
  source 1..124: note = VHH amino acid sequence of 7B11_huBSM_HM2
EVQLVESGGGLVQAGGSLRLSCAASGGTFLTYGMGWFRQAPGKEREFVAAINWSGSMTNYADSVKGRFTISRDNAKNTVYLQMRSLTSEDTAVYYCAAKTGAVAYIQKNEYDYWGQGTLVTVSS

SEQ ID NO: 85 - protein, 124 aa, synthetic construct
  source 1..124: note = VHH amino acid sequence of 7B11_huGS1
EVQLVESGGGLVQPGGSLRLSCAASGGTFLTYGMGWVRQAPGKGLEWVAAINWSGSMTNYADSVKGRFTISRDNAKNTVYLQMNSLRAEDTAVYYCAAKTGAVAYIQKNEYDYWGQGTLVTVSS

SEQ ID NO: 86 - protein, 124 aa, synthetic construct
  source 1..124: note = VHH amino acid sequence of 7B11_huGS_HM1
EVQLVESGGGLVQPGGSLRLSCAASGGTFLTYGMGWFRQAPGKGLEFVAAINWSGSMTNYADSVKGRFTISRDNAKNTVYLQMNSLRAEDTAVYYCAAKTGAVAYIQKNEYDYWGQGTLVTVSS

SEQ ID NO: 87 - protein, 124 aa, synthetic construct
  source 1..124: note = VHH amino acid sequence of 7B11_huGS_HM2
EVQLVESGGGLVQAGGSLRLSCAASGGTFLTYGMGWFRQAPGKGLEFVAAINWSGSMTNYADSVKGRFTISRDNAKNTVYLQMNSLRAEDTAVYYCAAKTGAVAYIQKNEYDYWGQGTLVTVSS

SEQ ID NO: 88 - protein, 124 aa, synthetic construct
  source 1..124: note = VHH amino acid sequence of 7B11_huGS_HM3
EVQLVESGGGLVQPGGSLRLSCAASGGTFLTYGMGWFRQAPGKEREFVAAINWSGSMTNYADSVKGRFTISRDNAKNTVYLQMNSLRAEDTAVYYCAAKTGAVAYIQKNEYDYWGQGTLVTVSS